European Patent Application EP 4 600 257 A1, published August 13, 2025. Title: A ribonuclease activity regulator protein variant and L-valine production method using same. Applicant: CJ CheilJedang Corporation. The sequence listing filed with the application follows.

SEQUENCE LISTING (14 sequences)

SEQ ID NO: 1 - protein, 168 aa, Corynebacterium glutamicum
MGMTQSAPEFIATADLVDIIGDNAQSCDTQFQNLGGATEFHGTITTVKCFQDNALLKSILSEDNPGGVLVIDGDASVHTALVGDIIAGLGKDHGWSGVIVNGAIRDSAVIGTMTFGCKALGTNPRKSTKTGSGERDVVVSIGGIDFIPGHYVYADSDGIIVTEAPIKQ

SEQ ID NO: 2 - DNA, 507 bp, Corynebacterium glutamicum
  source 1..507: mol_type = genomic DNA
gtgggcatgactcaaagtgctccagaattcattgccaccgcagacctcgtagacatcatcggcgacaacgcgcaatcatgcgacactcagtttcaaaaccttggaggtgccacagaattccacggaacaataaccaccgtgaaatgcttccaagacaacgccctcctgaaatccatcctgagcgaggataatcctgggggagtgctggttatcgacggcgacgcatccgtgcacaccgcgctagttggcgacatcattgcaggacttggaaaagatcatggttggtccggagtaattgtcaacggagcaattcgagactccgcagtcatcggcaccatgacctttggttgtaaagcccttggaaccaacccgcggaaatccactaaaactggttccggcgaacgagacgtagtggtatcgattggtggcattgacttcattcctggccattacgtctacgcggactctgacggaattatcgtcaccgaggcgccaattaagcagtaa

SEQ ID NO: 3 - protein, 168 aa, synthetic construct
MGMTQSAPEFIATADLVDIIGDNAQSCDTQFQNLGGATEFHGTITTVKCFQDNALLKSILSEDNPGGVLVIDGDASVHTALVGDIIAGLGKDYGWSGVIVNGAIRDSAVIGTMTFGCKALGTNPRKSTKTGSGERDVVVSIGGIDFIPGHYVYADSDGIIVTEAPIKQ

SEQ ID NO: 4 - DNA, 507 bp, synthetic construct
  source 1..507: mol_type = other DNA
gtgggcatgactcaaagtgctccagaattcattgccaccgcagacctcgtagacatcatcggcgacaacgcgcaatcatgcgacactcagtttcaaaaccttggaggtgccacagaattccacggaacaataaccaccgtgaaatgcttccaagacaacgccctcctgaaatccatcctgagcgaggataatcctgggggagtgctggttatcgacggcgacgcatccgtgcacaccgcgctagttggcgacatcattgcaggacttggaaaagattatggttggtccggagtaattgtcaacggagcaattcgagactccgcagtcatcggcaccatgacctttggttgtaaagcccttggaaccaacccgcggaaatccactaaaactggttccggcgaacgagacgtagtggtatcgattggtggcattgacttcattcctggccattacgtctacgcggactctgacggaattatcgtcaccgaggcgccaattaagcagtaa

SEQ ID NO: 5 - DNA, 27 bp, synthetic construct
  source 1..27: mol_type = other DNA
cccggggtgggcatgactcaaagtgct

SEQ ID NO: 6 - DNA, 27 bp, synthetic construct
  source 1..27: mol_type = other DNA
cccgggttactgcttaattggcgcctc

SEQ ID NO: 7 - DNA, 41 bp, synthetic construct
  source 1..41: mol_type = other DNA
cggggatcccccgggaggacggtactcaaatactaaacttc

SEQ ID NO: 8 - DNA, 38 bp, synthetic construct
  source 1..38: mol_type = other DNA
tgccgagtgtttcggtctttacagacacgagggacacg

SEQ ID NO: 9 - DNA, 31 bp, synthetic construct
  source 1..31: mol_type = other DNA
tgtctgtaaagaccgaaacactcggcatcaa

SEQ ID NO: 10 - DNA, 41 bp, synthetic construct
  source 1..41: mol_type = other DNA
cggggatcccccggggacaactacattattattataccaca

SEQ ID NO: 11 - DNA, 18 bp, synthetic construct
  source 1..18: mol_type = other DNA
ccgcgtcaccaaagcgga

SEQ ID NO: 12 - DNA, 20 bp, synthetic construct
  source 1..20: mol_type = other DNA
ttagatcttggccggagcca

SEQ ID NO: 13 - protein, 172 aa, synthetic construct
MANSDVTRHILSVLVQDVDGIISRVSGMFTRRAFNLVSLVSVKTETLGINRITVVVDADELNIEQITKQLNKLIPVLKVVRLDEETTIARAIMLVKVSADSTNRPQIVDAANIFRARVVDVAPDSVVIESTGTPGKLRALLDVMEPFGIRELIQSGQIALNRGPKTMAPAKI

SEQ ID NO: 14 - DNA, 519 bp, synthetic construct
  source 1..519: mol_type = other DNA
atggctaattctgacgtcacccgccacatcctgtccgtactcgttcaggacgtagacggaatcatttcccgcgtatcaggtatgttcacccgacgcgcattcaacctcgtgtccctcgtgtctgtaaagaccgaaacactcggcatcaaccgcatcacggttgttgtcgacgccgacgagctcaacattgagcagatcaccaagcagctcaacaagctgatccccgtgctcaaagtcgtgcgacttgatgaagagaccaccatcgcccgcgcaatcatgctggttaaggtctctgcggatagcaccaaccgtccgcagatcgtcgacgccgcgaacatcttccgcgcccgagtcgtcgacgtggctccagactctgtggttattgaatccacaggcaccccaggcaagctccgcgcactgcttgatgtgatggaaccattcggaatccgcgaactgatccaatccggacagattgcactcaaccgcggtccgaagaccatggctccggccaagatctaa